European Patent Specification EP 4 015 627 B1, published September 27, 2023. Title: CLOSTRIDIUM HISTOLYTICUM ENZYMES AND METHODS FOR THE USE THEREOF. Applicant: ENDO GLOBAL VENTURES. The sequence listing filed with the application follows.

SEQUENCE LISTING (30 sequences)

SEQ ID NO: 1 - DNA, 3357 bp, Clostridium histolyticum
atgaaaaaaaatattttaaagattcttatggatagttattctaaagaatctaaaattcaaactgtacgtagggttacgagtgtatcacttttagcggcatatcttactatgaatacttcaagtttagttttagcaaaaccaatagaaaatactaatgatactagtataaaaaatgtggagaaattaagaaatgctccaaatgaagagaatagtaaaaaggtagaagatagtaaaaatgataaggtagaacatgtggaaaatatagaagaggcaaaagttgagcaagttgcacccgaagtaaaatctaaatcaactttaagaagtgcttctatagcgaatactaattctgagaaatatgattttgagtatttaaatggtttgagctatactgaacttacaaatttaattaaaaatataaagtggaatcaaattaatggtttatttaattatagtacaggttctcaaaagttctttggagataaaaatcgtgtacaagctataattaatgctttacaagaaagtggaagaacttacactgcaaatgatatgaagggtatagaaactttcactgaggttttaagagctggtttttatttagggtactataatgatggtttatcttatttaaatgatagaaacttccaagataaatgtatacctgcaatgattgcaattcaaaaaaatcctaactttaagctaggaactgcagttcaagatgaagttataacttctttaggaaaactaataggaaatgcttctgctaatgctgaagtagttaataattgtgtaccagttctaaaacaatttagagaaaacttaaatcaatatgctcctgattacgttaaaggaacagctgtaaatgaattaattaaaggtattgaattcgatttttctggtgctgcatatgaaaaagatgttaagacaatgccttggtatggaaaaattgatccatttataaatgaacttaaggccttaggtctatatggaaatataacaagtgcaactgagtgggcatctgatgttggaatatactatttaagtaaattcggtctttactcaactaaccgaaatgacatagtacagtcacttgaaaaggctgtagatatgtataagtatggtaaaatagcctttgtagcaatggagagaataacttgggattatgatgggattggttctaatggtaaaaaggtggatcacgataagttcttagatgatgctgaaaaacattatctgccaaagacatatacttttgataatggaacctttattataagagcaggggagaaggtatccgaagaaaaaataaaaaggctatattgggcatcaagagaagtgaagtctcaattccatagagtagttggcaatgataaagctttagaggtgggaaatgccgatgatgttttaactatgaaaatatttaatagcccagaagaatataaatttaataccaatataaatggtgtaagcactgataatggtggtctatatatagaaccaagagggactttctacacttatgagagaacacctcaacaaagtatatttagtcttgaagaattgtttagacatgaatatactcactatttacaagcgagatatcttgtagatggtttatggggacaaggtccattttatgaaaaaaatagattaacttggtttgatgaaggtacagctgaattctttgcaggatctacccgtacatctggtgttttaccaagaaaatcaatattaggatatttggctaaggataaagtagatcatagatactcattaaagaagactcttaattcagggtatgatgacagtgattggatgttctataattatggatttgcagttgcacattatctatatgaaaaagatatgcctacatttattaagatgaataaagctatattgaatacagatgtgaaatcttatgatgaaataataaaaaaattaagtgatgatgcaaataaaaatacagaatatcaaaaccatattcaagagttagcagataaatatcaaggagcaggcatacctctagtatcagatgattacttaaaagatcatggatataagaaagcatctgaagtatattctgaaatttcaaaagctgcttctcttacaaacactagtgtaacagcagaaaaatctcaatattttaacacattcactttaagaggaacttatacaggtgaaacttctaaaggtgaatttaaagattgggatgaaatgagtaaaaaattagatggaactttggagtcccttgctaaaaattcttggagtggatacaaaactttaacagcatactttacgaattatagagttacaagcgataataaagttcaatatgatgtagttttccatggggttttaacagataatgcggatattagtaacaataaggctccaatagcaaaggtaactggaccaagcactggtgctgtaggaagaaatattgaatttagtggaaaagatagtaaagatgaagatggtaaaatagtatcatatgattgggattttggcgatggtgcaactagtagaggcaaaaattcagtacatgcttacaaaaaaacaggaacatataatgttacattaaaagtaactgacgataagggtgcaacagctacagaaagctttactatagaaataaagaacgaagatacaacaacacctataactaaagaaatggaacctaatgatgatataaaagaggctaatggtccaatagttgaaggtgttactgtaaaaggtgatttaaatggttctgatgatgctgataccttctattttgatgtaaaagaagatggtgatgttacaattgaacttccttattcagggtcatctaatttcacatggttagtttataaagagggagacgatcaaaaccatattgcaagtggtatagataagaataactcaaaagttggaacatttaaagctacaaaaggaagacattatgtgtttatatataaacacgattctgcttcaaatatatcctattctttaaacataaaaggattaggtaacgagaaattgaaggaaaaagaaaataatgattcttctgataaagctacagttataccaaatttcaataccactatgcaaggttcacttttaggtgatgattcaagagattattattcttttgaggttaaggaagaaggcgaagttaatatagaactagataaaaaggatgaatttggtgtaacatggacactacatccagagtcaaatattaatgacagaataacttacggacaagttgatggtaataaggtatctaataaagttaaattaagaccaggaaaatattatctacttgtttataaatactcaggatcaggaaactatgagttaagggtaaataaataa

SEQ ID NO: 2 - DNA, 3066 bp, Clostridium histolyticum
atgaaaaggaaatgtttatctaaaaggcttatgttagctataacaatggctacaatatttacagtgaacagtacattaccaatttatgcagctgtagataaaaataatgcaacagcagctgtacaaaatgaaagtaagaggtatacagtatcatatttaaagactttaaattattatgacttagtagatttgcttgttaagactgaaattgagaatttaccagacctttttcagtatagttcagatgcaaaagagttctatggaaataaaactcgtatgagctttatcatggatgaaattggtagaagggcaccacagtatacagagatagatcataaaggtattcctactttagtagaagttgtaagagctggattttacttaggattccataacaaggaattgaatgaaataaataagaggtcttttaaagaaagggtaataccttctatattggcaattcaaaaaaatcctaattttaaactaggtactgaagttcaagataaaatagtatctgcaacaggacttttagctggtaatgaaacagcgcctccagaagttgtaaataattttacaccaataattcaagactgtatcaaaaatatggacagatatgctcttgatgatttaaagtcaaaagcattatttaatgttttagctgcacctacctatgatataactgagtatttaagagctactaaagaaaaaccagaaaacactccttggtatggtaaaatagatgggtttataaatgaacttaaaaagttagctctttatggaaaaataaatgataataactcttggataatagataatggtatatatcatatagcacctttagggaagttacatagcaataataaaataggaatagaaactttaacagaggttatgaagatatatccttatttaagtatgcaacatttacaatcagcagatcaaattgagcgtcattatgattcaaaagatgctgaaggaaataaaatacctttagataagtttaaaaaggaaggaaaagagaaatactgtccaaaaacttatacatttgatgatggaaaagtaataataaaagctggtgctagggtagaagaagaaaaagttaaaagactatactgggcatcaaaggaagttaactctcaattctttagggtatatggaatagacaaaccattagaagaaggtaatccagatgatatattaacaatggttatctacaacagtcctgaagaatataaacttaatagtgttctatacggatatgatactaataatggtggtatgtatatagagccagatggaactttcttcacatatgaaagaaaagctgaagaaagcacatacacattagaagaattatttagacatgaatatacacactatttacaaggaagatatgcagttcctggtcaatggggaagaacaaaactttatgacaatgatagattaacttggtatgaagaaggtggagcagaattatttgcaggttctactagaacttctggaatattaccaagaaagagtatagtatcaaatattcataatacaacaagaaataatagatataagctttcagacactgtacattctaaatatggtgctagttttgaattctataattatgcatgtatgtttatggattatatgtataataaagatatgggtatattaaataaactaaatgatcttgcaaaaaataatgatgttgatggatatgataattatattagagatttaagttctaatcatgctttaaatgataaatatcaagatcatatgcaggagcgcatagataattatgaaaatttaacagtgccttttgtagctgatgattatttagtaagacatgcttataagaaccctaatgaaatttattctgaaatatctgaagtagcaaaattaaaggatgctaagagtgaagttaagaaatcacaatattttagtacctttactttgagaggtagttacacaggtggagcatctaaggggaaattagaagatcaaaaagcaatgaataagtttatagatgattcacttaagaaattagatacgtattcttggagtgggtataaaactttaactgcttatttcactaattataaagttgactcttcaaatagagttacttatgatgtagtattccacggatatttaccaaacgaaggtgattccaaaaattcattaccttatggcaagatcaatggaacttacaagggaacagagaaagaaaaaatcaaattctctagtgaaggctctttcgatccagatggtaaaatagtttcttatgaatgggatttcggagatggtaataagagtaatgaggaaaatccagagcattcatatgacaaggtaggaacttatacagtgaaattaaaagttactgatgacaagggagaatcttcagtatctactactactgcagaaataaaggatctttcagaaaataaacttccagttatatatatgcatgtacctaaatccggagccttaaatcaaaaagttgttttctatggaaaaggaacatatgacccagatggatctatcgcaggatatcaatgggactttggtgatggaagtgattttagcagtgaacaaaacccaagccatgtatatactaaaaaaggtgaatatactgtaacattaagagtaatggacagtagtggacaaatgagtgaaaaaactatgaagattaagattacagatccggtatatccaataggcactgaaaaagaaccaaataacagtaaagaaactgcaagtggtccaatagtaccaggtatacctgttagtggaaccatagaaaatacaagtgatcaagattatttctattttgatgttataacaccaggagaagtaaaaatagatataaataaattagggtacggaggagctacttgggtagtatatgatgaaaataataatgcagtatcttatgccactgatgatgggcaaaatttaagtggaaagtttaaggcagataaaccaggtagatattacatccatctttacatgtttaatggtagttatatgccatatagaattaatatagaaggttcagtaggaagataa

SEQ ID NO: 3 - protein, 1118 aa, Clostridium histolyticum
MKKNILKILMDSYSKESKIQTVRRVTSVSLLAAYLTMNTSSLVLAKPIENTNDTSIKNVEKLRNAPNEENSKKVEDSKNDKVEHVENIEEAKVEQVAPEVKSKSTLRSASIANTNSEKYDFEYLNGLSYTELTNLIKNIKWNQINGLFNYSTGSQKFFGDKNRVQAIINALQESGRTYTANDMKGIETFTEVLRAGFYLGYYNDGLSYLNDRNFQDKCIPAMIAIQKNPNFKLGTAVQDEVITSLGKLIGNASANAEVVNNCVPVLKQFRENLNQYAPDYVKGTAVNELIKGIEFDFSGAAYEKDVKTMPWYGKIDPFINELKALGLYGNITSATEWASDVGIYYLSKFGLYSTNRNDIVQSLEKAVDMYKYGKIAFVAMERITWDYDGIGSNGKKVDHDKFLDDAEKHYLPKTYTFDNGTFIIRAGEKVSEEKIKRLYWASREVKSQFHRVVGNDKALEVGNADDVLTMKIFNSPEEYKFNTNINGVSTDNGGLYIEPRGTFYTYERTPQQSIFSLEELFRHEYTHYLQARYLVDGLWGQGPFYEKNRLTWFDEGTAEFFAGSTRTSGVLPRKSILGYLAKDKVDHRYSLKKTLNSGYDDSDWMFYNYGFAVAHYLYEKDMPTFIKMNKAILNTDVKSYDEIIKKLSDDANKNTEYQNHIQELADKYQGAGIPLVSDDYLKDHGYKKASEVYSEISKAASLTNTSVTAEKSQYFNTFTLRGTYTGETSKGEFKDWDEMSKKLDGTLESLAKNSWSGYKTLTAYFTNYRVTSDNKVQYDVVFHGVLTDNADISNNKAPIAKVTGPSTGAVGRNIEFSGKDSKDEDGKIVSYDWDFGDGATSRGKNSVHAYKKTGTYNVTLKVTDDKGATATESFTIEIKNEDTTTPITKEMEPNDDIKEANGPIVEGVTVKGDLNGSDDADTFYFDVKEDGDVTIELPYSGSSNFTWLVYKEGDDQNHIASGIDKNNSKVGTFKATKGRHYVFIYKHDSASNISYSLNIKGLGNEKLKEKENNDSSDKATVIPNFNTTMQGSLLGDDSRDYYSFEVKEEGEVNIELDKKDEFGVTWTLHPESNINDRITYGQVDGNKVSNKVKLRPGKYYLLVYKYSGSGNYELRVNK

SEQ ID NO: 4 - protein, 1021 aa, Clostridium histolyticum
MKRKCLSKRLMLAITMATIFTVNSTLPIYAAVDKNNATAAVQNESKRYTVSYLKTLNYYDLVDLLVKTEIENLPDLFQYSSDAKEFYGNKTRMSFIMDEIGRRAPQYTEIDHKGIPTLVEVVRAGFYLGFHNKELNEINKRSFKERVIPSILAIQKNPNFKLGTEVQDKIVSATGLLAGNETAPPEVVNNFTPIIQDCIKNMDRYALDDLKSKALFNVLAAPTYDITEYLRATKEKPENTPWYGKIDGFINELKKLALYGKINDNNSWIIDNGIYHIAPLGKLHSNNKIGIETLTEVMKIYPYLSMQHLQSADQIERHYDSKDAEGNKIPLDKFKKEGKEKYCPKTYTFDDGKVIIKAGARVEEEKVKRLYWASKEVNSQFFRVYGIDKPLEEGNPDDILTMVIYNSPEEYKLNSVLYGYDTNNGGMYIEPDGTFFTYERKAEESTYTLEELFRHEYTHYLQGRYAVPGQWGRTKLYDNDRLTWYEEGGAELFAGSTRTSGILPRKSIVSNIHNTTRNNRYKLSDTVHSKYGASFEFYNYACMFMDYMYNKDMGILNKLNDLAKNNDVDGYDNYIRDLSSNHALNDKYQDHMQERIDNYENLTVPFVADDYLVRHAYKNPNEIYSEISEVAKLKDAKSEVKKSQYFSTFTLRGSYTGGASKGKLEDQKAMNKFIDDSLKKLDTYSWSGYKTLTAYFTNYKVDSSNRVTYDVVFHGYLPNEGDSKNSLPYGKINGTYKGTEKEKIKFSSEGSFDPDGKIVSYEWDFGDGNKSNEENPEHSYDKVGTYTVKLKVTDDKGESSVSTTTAEIKDLSENKLPVIYMHVPKSGALNQKVVFYGKGTYDPDGSIAGYQWDFGDGSDFSSEQNPSHVYTKKGEYTVTLRVMDSSGQMSEKTMKIKITDPVYPIGTEKEPNNSKETASGPIVPGIPVSGTIENTSDQDYFYFDVITPGEVKIDINKLGYGGATWVVYDENNNAVSYATDDGQNLSGKFKADKPGRYYIHLYMFNGSYMPYRINIEGSVGR

SEQ ID NO: 5 - protein, 1008 aa, Clostridium histolyticum
IANTNSEKYDFEYLNGLSYTELTNLIKNIKWNQINGLFNYSTGSQKFFGDKNRVQAIINALQESGRTYTANDMKGIETFTEVLRAGFYLGYYNDGLSYLNDRNFQDKCIPAMIAIQKNPNFKLGTAVQDEVITSLGKLIGNASANAEVVNNCVPVLKQFRENLNQYAPDYVKGTAVNELIKGIEFDFSGAAYEKDVKTMPWYGKIDPFINELKALGLYGNITSATEWASDVGIYYLSKFGLYSTNRNDIVQSLEKAVDMYKYGKIAFVAMERITWDYDGIGSNGKKVDHDKFLDDAEKHYLPKTYTFDNGTFIIRAGEKVSEEKIKRLYWASREVKSQFHRVVGNDKALEVGNADDVLTMKIFNSPEEYKFNTNINGVSTDNGGLYIEPRGTFYTYERTPQQSIFSLEELFRHEYTHYLQARYLVDGLWGQGPFYEKNRLTWFDEGTAEFFAGSTRTSGVLPRKSILGYLAKDKVDHRYSLKKTLNSGYDDSDWMFYNYGFAVAHYLYEKDMPTFIKMNKAILNTDVKSYDEIIKKLSDDANKNTEYQNHIQELADKYQGAGIPLVSDDYLKDHGYKKASEVYSEISKAASLTNTSVTAEKSQYFNTFTLRGTYTGETSKGEFKDWDEMSKKLDGTLESLAKNSWSGYKTLTAYFTNYRVTSDNKVQYDVVFHGVLTDNADISNNKAPIAKVTGPSTGAVGRNIEFSGKDSKDEDGKIVSYDWDFGDGATSRGKNSVHAYKKTGTYNVTLKVTDDKGATATESFTIEIKNEDTTTPITKEMEPNDDIKEANGPIVEGVTVKGDLNGSDDADTFYFDVKEDGDVTIELPYSGSSNFTWLVYKEGDDQNHIASGIDKNNSKVGTFKATKGRHYVFIYKHDSASNISYSLNIKGLGNEKLKEKENNDSSDKATVIPNFNTTMQGSLLGDDSRDYYSFEVKEEGEVNIELDKKDEFGVTWTLHPESNINDRITYGQVDGNKVSNKVKLRPGKYYLLVYKYSGSGNYELRVNK

SEQ ID NO: 6 - protein, 991 aa, Clostridium histolyticum
AVDKNNATAAVQNESKRYTVSYLKTLNYYDLVDLLVKTEIENLPDLFQYSSDAKEFYGNKTRMSFIMDEIGRRAPQYTEIDHKGIPTLVEVVRAGFYLGFHNKELNEINKRSFKERVIPSILAIQKNPNFKLGTEVQDKIVSATGLLAGNETAPPEVVNNFTPIIQDCIKNMDRYALDDLKSKALFNVLAAPTYDITEYLRATKEKPENTPWYGKIDGFINELKKLALYGKINDNNSWIIDNGIYHIAPLGKLHSNNKIGIETLTEVMKIYPYLSMQHLQSADQIERHYDSKDAEGNKIPLDKFKKEGKEKYCPKTYTFDDGKVIIKAGARVEEEKVKRLYWASKEVNSQFFRVYGIDKPLEEGNPDDILTMVIYNSPEEYKLNSVLYGYDTNNGGMYIEPDGTFFTYERKAEESTYTLEELFRHEYTHYLQGRYAVPGQWGRTKLYDNDRLTWYEEGGAELFAGSTRTSGILPRKSIVSNIHNTTRNNRYKLSDTVHSKYGASFEFYNYACMFMDYMYNKDMGILNKLNDLAKNNDVDGYDNYIRDLSSNHALNDKYQDHMQERIDNYENLTVPFVADDYLVRHAYKNPNEIYSEISEVAKLKDAKSEVKKSQYFSTFTLRGSYTGGASKGKLEDQKAMNKFIDDSLKKLDTYSWSGYKTLTAYFTNYKVDSSNRVTYDVVFHGYLPNEGDSKNSLPYGKINGTYKGTEKEKIKFSSEGSFDPDGKIVSYEWDFGDGNKSNEENPEHSYDKVGTYTVKLKVTDDKGESSVSTTTAEIKDLSENKLPVIYMHVPKSGALNQKVVFYGKGTYDPDGSIAGYQWDFGDGSDFSSEQNPSHVYTKKGEYTVTLRVMDSSGQMSEKTMKIKITDPVYPIGTEKEPNNSKETASGPIVPGIPVSGTIENTSDQDYFYFDVITPGEVKIDINKLGYGGATWVVYDENNNAVSYATDDGQNLSGKFKADKPGRYYIHLYMFNGSYMPYRINIEGSVGR

SEQ ID NO: 7 - protein, 443 aa, Clostridium septicum
MSKKSFAKKVICTSMIAIQCAAVVPHVQAYALTNLEEGGYANHNNASSIKIFGYEDNEDLKAKIIQDPEFIRNWANVAHSLGFGWCGGTANPNVGQGFEFKREVGAGGKVSYLLSARYNPNDPYASGYRAKDRLSMKISNVRFVIDNDSIKLGTPKVKKLAPLNSASFDLINESKTESKLSKTFNYTTSKTVSKTDNFKFGEKIGVKTSFKVGLEAIADSKVETSFEFNAEQGWSNTNSTTETKQESTTYTATVSPQTKKRLFLDVLGSQIDIPYEGKIYMEYDIELMGFLRYTGNAREDHTEDRPTVKLKFGKNGMSAEEHLKDLYSHKNINGYSEWDWKWVDEKFGYLFKNSYDALTSRKLGGIIKGSFTNINGTKIVIREGKEIPLPDKKRRGKRSVDSLDARLQNEGIRIENIETQDVPGFRLNSITYNDKKLILINNI

SEQ ID NO: 8 - protein, 419 aa, Clostridium histolyticum
MLKKSFFKKAICASLVVLQCLILVSPAQTLASTDLPTKGKTSIELFNYEDHMAHCLGFGWCFGTASKEIGEDFEFKRAEEEGKTVYYLSARYNQNDPYAKGYYRAHDRLVMKVSNARFFIDHDSLTLGKAKVISLDPLASSTLQVVNKSNSEAKTSLSFGYETTESTSKTDHVKFGEKIGIKSSFNVKVPFIGEKSIETNLEFNSEQGWSNTKTNSVTTKHTISHTTTTPAKSRKKVRLNVLNKKSDIPYEGKIYMEYDIEFFGFLRYTGNARKDHPTDRPSVSVKFGGKNNMSAVDHIIDLYKHKDINGYSEWDWNWIEENFYDRFSEYSSNVASQYFGGIISGVFTNVGGTDVKVEEGRERPLKNTSSTEQNVEVQNFKSSKSKEFRVGSLTYTTPNGEQTIYPEDVSSLNANNNEN

SEQ ID NO: 9 - protein, 548 aa, Bacillus proteolyticus
MKMKMKLASFGLAAGLAAQVFLPYNALASTEHVTWNQQFQTPQFISGDLLKVNGTSPEELVYQYVEKNENKFKFHENAKDTLQLKEKKNDNLGFTFMRFQQTYKGIPVFGAVVTSHVKDGTLTALSGTLIPNLDTKGSLKSGKKLSEKQARDIAEKDLVANVTKEVPEYEQGKDTEFVVYVNGDEASLAYVVNLNFLTPEPGNWLYIIDAVDGKILNKFNQLDAAKPGDVKSITGTSTVGVGRGVLGDQKNINTTYSTYYYLQDNTRGNGIFTYDAKYRTTLPGSLWADADNQFFASYDAPAVDAHYYAGVTYDYYKNVHNRLSYDGNNAAIRSSVHYSQGYNNAFWNGSQMVYGDGDGQTFIPLSGGIDVVAHELTHAVTDYTAGLIYQNESGAINEAISDIFGTLVEFYANKNPDWEIGEDVYTPGISGDSLRSMSDPAKYGDPDHYSKRYTGTQDNGGVHINSGIINKAAYLISQGGTHYGVSVVGIGRDKLGKIFYRALTQYLTPTSNFSQLRAAAVQSATDLYGSTSQEVASVKQAFDAVGVK

SEQ ID NO: 10 - protein, 532 aa, Clostridium histolyticum
MKKKFLSFIIISAISLNISSMTVGAKQVKEIKPPKDKESISVLKTDLEKTKNIKSNNKEGDDVTKVVKSALKEEGNLGDFKVDNKETDVKGKKHLRSQMFIDGIPVYGSQVIIHTNKDGQVYSVNGKVDKQPKAQSFKNRVRIKDDKAIKIAEDSLGKEIKKNKNYHSESKLYLYKVNGDLQPVYLVKISSTEPEASFWHMFVSAENGKIVDKYNALSCQATHAQVRGVNSSGEHKILNGMFENGRYFLADSTRPSNGYILTYDANNQEYGFPGSLFSNLTGIFDSDRQKAGVDAHHNLTQVYDYYKNVLNRDSFDGKGASIISSVHVGNNLNNAFWNGRQILFGDGDGVTFSNLAKCLEVTAHEFTHAVTQSTAGLEYRFQSGALNEAFSDILGIAVHSDPNDWEIGEDIYTPNVAGDALRSMSNPRLYRQPDHMKDYLYWDYSMDKGGVHYNSGIPNKAAYLMGKEVGKDSMAKIYYHALVNYLTPQSTFEDARNAVVSSAIDLHGENSKEHKLAIKSWADVGVGEEAVR

SEQ ID NO: 11 - protein, 204 aa, Bacillus proteolyticus
STEHVTWNQQFQTPQFISGDLLKVNGTSPEELVYQYVEKNENKFKFHENAKDTLQLKEKKNDNLGFTFMRFQQTYKGIPVFGAVVTSHVKDGTLTALSGTLIPNLDTKGSLKSGKKLSEKQARDIAEKDLVANVTKEVPEYEQGKDTEFVVYVNGDEASLAYVVNLNFLTPEPGNWLYIIDAVDGKILNKFNQLDAAKPGDVKS

SEQ ID NO: 12 - protein, 194 aa, Clostridium histolyticum
KPPKDKESISVLKTDLEKTKNIKSNNKEGDDVTKVVKSALKEEGNLGDFKVDNKETDVKGKKHLRSQMFIDGIPVYGSQVIIHTNKDGQVYSVNGKVDKQPKAQSFKNRVRIKDDKAIKIAEDSLGKEIKKNKNYHSESKLYLYKVNGDLQPVYLVKISSTEPEASFWHMFVSAENGKIVDKYNALSCQATHAQ

SEQ ID NO: 13 - protein, 316 aa, Bacillus proteolyticus
ITGTSTVGVGRGVLGDQKNINTTYSTYYYLQDNTRGNGIFTYDAKYRTTLPGSLWADADNQFFASYDAPAVDAHYYAGVTYDYYKNVHNRLSYDGNNAAIRSSVHYSQGYNNAFWNGSQMVYGDGDGQTFIPLSGGIDVVAHELTHAVTDYTAGLIYQNESGAINEAISDIFGTLVEFYANKNPDWEIGEDVYTPGISGDSLRSMSDPAKYGDPDHYSKRYTGTQDNGGVHINSGIINKAAYLISQGGTHYGVSVVGIGRDKLGKIFYRALTQYLTPTSNFSQLRAAAVQSATDLYGSTSQEVASVKQAFDAVGVK

SEQ ID NO: 14 - protein, 307 aa, Clostridium histolyticum
VRGVNSSGEHKILNGMFENGRYFLADSTRPSNGYILTYDANNQEYGFPGSLFSNLTGIFDSDRQKAGVDAHHNLTQVYDYYKNVLNRDSFDGKGASIISSVHVGNNLNNAFWNGRQILFGDGDGVTFSNLAKCLEVTAHEFTHAVTQSTAGLEYRFQSGALNEAFSDILGIAVHSDPNDWEIGEDIYTPNVAGDALRSMSNPRLYRQPDHMKDYLYWDYSMDKGGVHYNSGIPNKAAYLMGKEVGKDSMAKIYYHALVNYLTPQSTFEDARNAVVSSAIDLHGENSKEHKLAIKSWADVGVGEEAVR

SEQ ID NO: 15 - protein, 500 aa, Clostridium perfringens
MIRFKKTKLIASIAMALCLFSQPVISFSKDITDKNQSIDSGISSLSYNRNEVLASNGDKIESFVPKEGKKTGNKFIVVERQKRSLTTSPVDISIIDSVNDRTYPGALQLADKAFVENRPTILMVKRKPININIDLPGLKGENSIKVDDPTYGKVSGAIDELVSKWNEKYSSTHTLPARTQYSESMVYSKSQISSALNVNAKVLENSLGVDFNAVANNEKKVMILAYKQIFYTVSADLPKNPSDLFDDSVTFNDLKQKGVSNEAPPLMVSNVAYGRTIYVKLETTSSSKDVQAAFKALIKNTDIKNSQQYKDIYENSSFTAVVLGGDAQEHNKVVTKDFDEIRKVIKDNATFSTKNPAYPISYTSVFLKDNSVAAVHNKTDYIETTSTEYSKGKINLDHSGAYVAQFEVAWDEVSYDKEGNEVLTHKTWDGNYQDKTAHYSTVIPLEANARNIRIKARECTGLAWEWWRDVISEYDVPLTNNINVSIWGTTLYPGSSITYN

SEQ ID NO: 16 - protein, 520 aa, Clostridium histolyticum
MKITKKGLRSLSRLMLITMITGLTYNYHLGSSFNGNRVVLANPNTKTDNLIKNNSDEIDEKIYGLSYDPYKILSYNGEKVENFVPAECSENSGKFTVIKREKKNISDSTTDISIMDSINDRTYPGAIQLANRDLIENKPNLISCERKPITISVDLPGMGEDGKKVVNSPTYSSVNSAINYLLDTWNSKYSSKYTIPTRMNYSDTMVYSKSQLSTMFGCNFKTLSKSLNIDFDSIFKGEKKAMILSYKQIFYTVSVDGPNRPSDLFGYSVTSKSLALKGVNNDNPPAYVSNVAYGRTVYVKLETTSKSSKVKAAFKALVENQDISSNAEYKDIINQSSFTATVLGGGAQKHNKVVTKDFDVIRNIIKNNSVYSPQNPGYPISYTSTFLKDNKIATVNNRTEYIETTATEYDSGKIMLDHSGVYVAQFEVTWDEVSYDKQGNEIIEHKSWSGNNSDRTAHFNTELYLKGNARNISIKAKECTGLAWEWWRTVVDAKNLPLVKERKLSIWGTTLYPRYSMEEK

SEQ ID NO: 17 - protein, 526 aa, Clostridium histolyticum
MLRRKVSTLLMTALITTSFLNSKPVYANPVTKSKDNNLKEVQQVTSKSNKNKNQKVTIMYYCDADNNLEGSLLNDIEEMKTGYKDSPNLNLIALVDRSPRYSSDEKVLGEDFSDTRLYKIEHNKANRLDGKNEFPEISTTSKYEANMGDPEVLKKFIDYCKSNYEADKYVLIMANHGGGAREKSNPRLNRAICWDDSNLDKNGEADCLYMGEISDHLTEKQSVDLLAFDACLMGTAEVAYQYRPGNGGFSADTLVASSPVVWGPGFKYDKIFDRIKAGGGTNNEDDLTLGGKEQNFDPATITNEQLGALFVEEQRDSTHANGRYDQHLSFYDLKKAESVKRAIDNLAVNLSNENKKSEIEKLRGSGIHTDLMHYFDEYSEGEWVEYPYFDVYDLCEKINKSENFSSKTKDLASNAMNKLNEMIVYSFGDPSNNFKEGKNGLSIFLPNGDKKYSTYYTSTKIPHWTMQSWYNSIDTVKYGLNPYGKLSWCKDGQDPEINKVGNWFELLDSWFDKTNDVTGGVNHYQW

SEQ ID NO: 18 - protein, 526 aa, Clostridium histolyticum
MLRRKVSTLLMTALITTSFLNSKPVYANPVTKSKDNNLKEVQQVISKSNKNKNQKVTIMYYCDADNNLEGSLLNDIEEMKTGYKDSPNLNLIALVDRSPRYSSDEKVLGEDFSDTRLYKIELNKANRLDGKNEFPEISTTSKYEANMGDPEVLKKFIDYCKSNYEADKYVLIMANHGGGAREKSNPRLNRAICWDDSNLDKNGEADCLYMGEISDHLTEKQSVDLLAFDACLMGTAEVAYQYRPGNGGFSADTLVASSPVVWGPGFKYDKIFDRIKAGGGTNNEDDLTLGGKEQNFDPATITNEQLGALFVEEQRDSTHANGRYDQHLSFYDLKKAESVKRAIDNLAVNLSNENKKSEIEKLRGSGIHTDLMHYFDEYSEGEWVEYPYFDVYDLCEKINKSENFSSKTKDLASNAMNKLNEMIVYSFGDPSNNFKEGKNGLSTFLPNGDKKYSTYYTSTKIPHWTMQSWYNSIDTVKYGLNPYGKLSWCKDGQDPEINKVGNWFELLDSWFDKTNDVTGGVNHYQW

SEQ ID NO: 19 - protein, 1118 aa, Clostridium histolyticum
MKKNILKILMDSYSKESKIQTVRRVTSVSLLAVYLTMNTSSLVLAKPIENTNDTSIKNVEKLRNAPNEENSKKVEDSKNDKVEHVKNIEEAKVEQVAPEVKSKSTLRSASIANTNSEKYDFEYLNGLSYTELTNLIKNIKWNQINGLFNYSTGSQKFFGDKNRVQAIINALQESGRTYTANDMKGIETFTEVLRAGFYLGYYNDGLSYLNDRNFQDKCIPAMIAIQKNPNFKLGTAVQDEVITSLGKLIGNASANAEVVNNCVPVLKQFRENLNQYAPDYVKGTAVNELIKGIEFDFSGAAYEKDVKTMPWYGKIDPFINELKALGLYGNITSATEWASDVGIYYLSKFGLYSTNRNDIVQSLEKAVDMYKYGKIAFVAMERITWDYDGIGSNGKKVDHDKFLDDAEKHYLPKTYTFDNGTFIIRAGDKVSEEKIKRLYWASREVKSQFHRVVGNDKALEVGNADDVLTMKIFNSPEEYKFNTNINGVSTDNGGLYIEPRGTFYTYERTPQQSIFSLEELFRHEYTHYLQARYLVDGLWGQGPFYEKNRLTWFDEGTAEFFAGSTRTSGVLPRKSILGYLAKDKVDHRYSLKKTLNSGYDDSDWMFYNYGFAVAHYLYEKDMPTFIKMNKAILNTDVKSYDEIIKKLSDDANKNTEYQNHIQELADKYQGAGIPLVSDDYLKDHGYKKASEVYSEISKAASLTNTSVTAEKSQYFNTFTLRGTYTGETSKGEFKDWDEMSKKLDGTLESLAKNSWSGYKTLTAYFTNYRVTSDNKVQYDVVFHGVLTDNADISNNKAPIAKVTGPSTGAVGRNIEFSGKDSKDEDGKIVSYDWDFGDGATSRGKNSVHAYKKAGTYNVTLKVTDDKGATATESFTIEIKNEDTTTPITKEMEPNDDIKEANGPIVEGVTVKGDLNGSDDADTFYFDVKEDGDVTIELPYSGSSNFTWLVYKEGDDQNHIASGIDKNNSKVGTFKSTKGRHYVFIYKHDSASNISYSLNIKGLGNEKLKEKENNDSSDKATVIPNFNTTMQGSLLGDDSRDYYSFEVKEEGEVNIELDKKDEFGVTWTLHPESNINDRITYGQVDGNKVSNKVKLRPGKYYLLVYKYSGSGNYELRVNK

SEQ ID NO: 20 - protein, 1021 aa, Clostridium histolyticum
MKRKCLSKRLMLAITMATIFTVNSTLPIYAAVDKNNATAAVQNESKRYTVSYLKTLNYYDLVDLLVKTEIENLPDLFQYSSDAKEFYGNKTRMSFIMDEIGRRAPQYTEIDHKGIPTLVEVVRAGFYLGFHNKELNEINKRSFKERVIPSILAIQKNPNFKLGTEVQDKIVSATGLLAGNETAPPEVVNNFTPILQDCIKNIDRYALDDLKSKALFNVLAAPTYDITEYLRATKEKPENTPWYGKIDGFINELKKLALYGKINDNNSWIIDNGIYHIAPLGKLHSNNKIGIETLTEVMKVYPYLSMQHLQSADQIKRHYDSKDAEGNKIPLDKFKKEGKEKYCPKTYTFDDGKVIIKAGARVEEEKVKRLYWASKEVNSQFFRVYGIDKPLEEGNPDDILTMVIYNSPEEYKLNSVLYGYDTNNGGMYIEPEGTFFTYEREAQESTYTLEELFRHEYTHYLQGRYAVPGQWGRTKLYDNDRLTWYEEGGAELFAGSTRTSGILPRKSIVSNIHNTTRNNRYKLSDTVHSKYGASFEFYNYACMFMDYMYNKDMGILNKLNDLAKNNDVDGYDNYIRDLSSNYALNDKYQDHMQERIDNYENLTVPFVADDYLVRHAYKNPNEIYSEISEVAKLKDAKSEVKKSQYFSTFTLRGSYTGGASKGKLEDQKAMNKFIDDSLKKLDTYSWSGYKTLTAYFTNYKVDSSNRVTYDVVFHGYLPNEGDSKNSLPYGKINGTYKGTEKEKIKFSSEGSFDPDGKIVSYEWDFGDGNKSNEENPEHSYDKVGTYTVKLKVTDDKGESSVSTTTAEIKDLSENKLPVIYMHVPKSGALNQKVVFYGKGTYDPDGSIAGYQWDFGDGSDFSSEQNPSHVYTKKGEYTVTLRVMDSSGQMSEKTMKIKITDPVYPIGTEKEPNNSKETASGPIVPGIPVSGTIENTSDQDYFYFDVITPGEVKIDINKLGYGGATWVVYDENNNAVSYATDDGQNLSGKFKADKPGRYYIHLYMFNGSYMPYRINIEGSVGR

SEQ ID NO: 21 - DNA, 1263 bp, Clostridium histolyticum
atgttaaaaaaatctttttttaaaaaggcaatttgcgcatctttggtggtgctacaatgtttgatattagtgtcaccagctcaaacattggcatcaacagatttgccgacaaaaggaaaaacttcaattgaactatttaactatgaagatcattaaatggctcattgtttgggatttggatggtgcttcggtacagcatcaaaagaaataggggaagattttgaatttaaaagagcagaagaagaaggaaaaacagtatattatttatcagctagatacaatcaaaatgatccttacgctaaaggctattatcgcgcgcatgataggcttgttatgaaggttagtaatgctaggttttttatcgatcatgattcattaactttaggaaaagctaaagttataagtctagatccactggcatcatcaactcttcaagtagtaaataaaagtaattctgaagctaaaacatcattatcttttggatatgaaactactgaaagtacttccaaaacggatcacgttaaattcggagaaaaaattggaattaagtcatcatttaatgttaaagttccatttataggagaaaaatcaattgaaacaaatcttgaattcaattcagagcagggttggtccaatacgaaaactaactctgtaactactaaacatacaatttctcatacaacaacaacacctgcaaagagcaggaaaaaggtacgattaaatgttcttaataaaaagtccgacataccatatgagggtaagatatatatggaatatgatatagagttttttggttttttaagatatactggaaatgcgcgtaaagatcatcctacagatagacctagtgtatcagtaaaatttgggggaaaaaataatatgagtgcggtagatcatattatagatttgtacaagcataaagatattaatggctattcagaatgggattggaattggattgaagaaaatttttatgatagatttagtgaatattcatctaatgttgctagtcaatattttgggggcattatttctggtgtatttactaatgtgggtggaacagatgtaaaagttgaagaaggtagagaaaggccacttaaaaatacaagttctacagaacaaaatgtcgaagtacagaattttaaaagctctaaatctaaagagtttagagtgggtagtttaacatatactactcctaatggagaacagaccatatatcctgaagacgtatcatctcttaacgctaacaacaatgagaattaa

SEQ ID NO: 22 - DNA, 1599 bp, Clostridium histolyticum
atgaaaaaaaaatttttaagttttattattatttctgccatatcacttaacatttcttctatgactgtgggggcaaagcaagtgaaagaaatcaaacctccaaaagataaagaatctatttctgtattaaaaacagatttagaaaaaaccaagaatataaaatctaataataaggagggggatgatgtaacaaaagtagttaagagtgctttaaaagaagaaggcaatttaggagattttaaggttgataataaagaaactgatgtaaaaggtaaaaagcacttgcgttcacaaatgtttatagatggtattcctgtatatggtagtcaagttataattcatactaataaagatggacaagtatatagcgtaaatggaaaagtagataaacagcctaaagctcaatcttttaagaaccgtgtaaggattaaggacgataaagctattaaaatagcagaagacagtttaggtaaggaaataaagaaaaacaaaaattatcattctgaaagtaagttgtacctatacaaggttaatggagatttacaacctgtgtatttggtaaagatatcatctacagaaccagaagcttcattttggcatatgtttgtaagtgctgaaaatggaaagatagttgataagtataatgctttatcatgccaagctacacatgctcaagtaagaggagttaatagcagtggagagcataaaatcttaaatggtatgtttgaaaatggaagatattttttagcagattcaacaagaccttcaaatggatatatattaacatatgatgctaataaccaagagtatggtttcccaggtagcttatttagtaatttaacaggcatttttgatagtgatagacaaaaggcaggagtagatgctcaccataatctaactcaagtatatgattattataaaaatgttttaaatagagatagttttgatggaaaaggtgctagtataatatcttctgtgcatgtaggaaataatttaaataatgctttctggaatggtagacaaatactttttggtgatggagacggagttacatttagtaacctagcaaaatgtttagaagttactgcccatgaatttacacatgcagttactcaaagtactgcaggtctagaatatagatttcaatctggtgctctaaatgaagctttttctgatattttaggtatagctgttcacagtgatccaaatgattgggaaattggagaagatatatacactcctaatgtagcaggagatgctttaagaagtatgtcaaatcctagattatatagacaaccagaccatatgaaggactatttatattgggattattcaatggataaaggtggagttcattataattcaggtattccaaataaagcagcttatttgatgggaaaagaagttggaaaagattcaatggctaaaatttattatcatgctttagtgaattatttaactcctcaaagtacatttgaagatgctagaaatgcagtagtatcatctgcaatagatttacatggtgagaatagtaaagaacataaacttgctataaaatcttgggcagatgtaggcgttggagaagaggcagtaagataa

SEQ ID NO: 23 - DNA, 1563 bp, Clostridium histolyticum
atgaagattacaaagaaaggcttaagatcattatcacgcttaatgttaattactatgataacaggattaacatacaattatcacctaggtagtagctttaatgggaatcgagtagtacttgcaaatccaaatacaaaaacagataatttaattaagaataatagtgatgaaatagacgaaaagatttatggattgtcttatgatccatataaaatattatcttataatggagaaaaggttgaaaactttgttccagctgaatgttccgagaattccggaaaatttactgtaataaaacgtgaaaagaaaaatatttcagattcaactacagatatttcaataatggattcaataaatgatagaacttatcctggtgctatacaactagcaaatagggatcttatagaaaataagcctaatttaatttcatgcgagagaaaacctattactataagtgttgatttacctggtatgggtgaggatgggaaaaaggttgttaattctccaacatactcttcagttaattcagcaataaattatttgctagatacatggaattcaaaatattcatctaaatatactatacctacaaggatgaattattctgatactatggtgtatagtaaatcacagttatctacaatgtttggatgtaactttaaaactttaagtaaatccttaaatatagattttgattctatatttaaaggcgaaaaaaaggctatgattctatcatataaacaaattttctacacagtgagtgtagatggacctaatcgcccatcagatttatttggttacagtgtaacttctaagagcttagctttaaaaggagtaaataatgataatcctccagcatacgtttccaatgttgcatatggtagaactgtttatgtaaaactagagacaacatctaagagttcaaaggttaaagcagcatttaaggcattagtagagaatcaagatataagtagtaatgcagaatataaagacataataaatcaaagttcatttacagctactgttctaggtggaggagcacaaaaacacaataaagtagttactaaagatttcgatgtaataagaaatattattaaaaataattcagtatatagcccacaaaatcctggatatcctatttcatatacaagtacatttttaaaagacaataaaatagcaactgtaaacaatagaacagaatatatagaaacaactgcaacagaatacgatagcggcaaaataatgcttgaccatagtggagtttatgttgctcaatttgaagtaacctgggatgaagttagttatgacaaacaaggaaatgaaataattgagcataaatcttggtctggaaacaatagtgatagaacagctcactttaatacagaactatatttaaaaggaaatgcaagaaacatttctataaaagcaaaagaatgtacaggccttgcttgggaatggtggagaactgttgtagatgctaaaaatttaccacttgtaaaagaaagaaagttatcaatatggggtacaacattatatcctagatattctatggaagagaaataa

SEQ ID NO: 24 - DNA, 1581 bp, Clostridium histolyticum
atgttaagaagaaaagtatcaacactattaatgacagctttgataactacttcatttttaaattccaaacccgtatatgcaaatccagtaactaaatccaaggataataacttaaaagaagtacaacaagttataagcaagagtaataaaaacaaaaatcaaaaagtaactattatgtactattgcgacgcagataataacttggaaggaagtctattaaatgatatcgaggaaatgaaaacaggatataaggatagtcctaatttaaatttaattgctcttgtagacagatccccaagatatagcagtgacgaaaaagttttaggtgaagattttagtgatacacgtctttataagattgaactcaataaggcaaatagattagacggtaaaaatgaatttccagaaataagtactactagtaaatatgaagctaacatgggggatcctgaagttcttaaaaaatttattgattattgtaaatctaattatgaggctgataaatatgtgcttataatggctaatcatggtggtggtgcaagggaaaaatcaaatccaagattaaatagagcaatttgctgggatgatagtaaccttgataaaaatggtgaagcagactgcctttatatgggtgaaatttcagatcatttaacagaaaaacaatcagttgatttacttgcctttgatgcatgccttatgggaactgcagaagtagcgtatcagtatagaccaggtaatggaggattttctgccgatactttagttgcttcaagcccagtagtttggggtcctggattcaaatatgataagattttcgataggataaaagctggtggaggaactaataatgaggatgatttaactttaggtggtaaagaacaaaactttgatcctgcaaccattaccaatgagcaattaggtgcattatttgtagaagagcaaagagactcaacacatgccaatggtcgctatgatcaacacttaagcttttatgatttaaagaaagctgaatcagtaaaaagagccatagataatttagctgttaatctaagtaatgaaaacaaaaaatctgaaattgaaaaattaagaggaagtggaattcatacagatttaatgcattacttcgatgaatattctgaaggagaatgggttgaatatccttattttgacgtgtatgatttatgtgaaaaaataaataaaagtgaaaattttagtagtaaaactaaagatttagcttcaaatgctatgaataaattaaatgaaatgatagtttattcttttggagaccctagtaataattttaaagaaggaaaaaatggattgagtacattcttacctaatggagataaaaaatattcaacttattatacatcaaccaagatacctcattggactatgcaaagttggtataattcaatagatacagttaaatatggattgaatccttacggaaaattaagttggtgtaaagatggacaagatcctgaaataaataaagttggaaattggtttgaacttctagattcttggtttgataaaactaatgatgtaactggaggagttaatcattaccaatggtaa

SEQ ID NO: 25 - protein, 6 aa, Artificial Sequence
  Description of Artificial Sequence: Synthetic 6xHis tag
HHHHHH

SEQ ID NO: 26 - protein, 12 aa, Clostridium septicum
DKKRRGKRSVDS

SEQ ID NO: 27 - protein, 11 aa, Clostridium histolyticum
NTSSTEQNVEV

SEQ ID NO: 28 - protein, 10 aa, Bacillus proteolyticus
AHELTHAVTD

SEQ ID NO: 29 - protein, 11 aa, Clostridium perfringens
ECTGLAWEWWR

SEQ ID NO: 30 - protein, 4 aa, Clostridium histolyticum
AVDK